European Patent Application EP 4 356 931 A1, published April 24, 2024. Title: PRPF31 VARIANT AND USES THEREOF. Applicant: Chigenovo Co., Ltd. The sequence listing filed with the application follows.

SEQUENCE LISTING (36 sequences)

SEQ ID NO: 1 - protein, 7 aa, Artificial Sequence
  sv40
PKKKRKV

SEQ ID NO: 2 - protein, 20 aa, Artificial Sequence
  hnRNPA1
SSNFGPMKGGNRFFRSSGPY

SEQ ID NO: 3 - protein, 12 aa, Artificial Sequence
  HIV Tat
GRKKRRQRRRAP

SEQ ID NO: 4 - protein, 27 aa, Artificial Sequence
  hnRNPD
YGDYSNQQSGYGKVSRRGGHQNSYKPY

SEQ ID NO: 5 - protein, 26 aa, Artificial Sequence
  hnRNPM
GEGERPAQNEKRKENIKRGGNRFEPY

SEQ ID NO: 6 - protein, 16 aa, Artificial Sequence
  nuleoplasmin
KRPAATKKAGQAKKKK

SEQ ID NO: 7 - protein, 19 aa, Artificial Sequence
  SRY
HREKYPNYKYRPRRKAKML

SEQ ID NO: 8 - DNA, 21 bp, Artificial Sequence
  sv40
cctaagaagaaaagaaaggtg

SEQ ID NO: 9 - DNA, 60 bp, Artificial Sequence
  hnRNPA1
tctagcaacttcggccctatgaagggcggaaaccggttctttagaagctccggcccctac

SEQ ID NO: 10 - DNA, 36 bp, Artificial Sequence
  HIV Tat
ggcagaaagaagcggagacagagaagacgggcccct

SEQ ID NO: 11 - DNA, 81 bp, Artificial Sequence
  hnRNPD
tatggcgactacagcaaccagcagtccggctacggcaaggtgtctagacggggcggacaccagaacagctacaagccttac

SEQ ID NO: 12 - DNA, 78 bp, Artificial Sequence
  hnRNPM
ggcgaaggcgagagacctgcccagaacgagaaaagaaaggaaaacatcaagcggggcggaaatagattcgagccctac

SEQ ID NO: 13 - DNA, 48 bp, Artificial Sequence
  nuleoplasmin
aaaagacctgctgccaccaagaaggccggccaggccaagaagaaaaag

SEQ ID NO: 14 - DNA, 57 bp, Artificial Sequence
  SRY
cacagagagaaataccccaactacaagtaccggcctagaagaaaggccaagatgctg

SEQ ID NO: 15 - protein, 14 aa, Artificial Sequence
  Nuclear localization signal sequence of PRPF31 protein
RKKRGGRRYRKMKE

SEQ ID NO: 16 - DNA, 42 bp, Artificial Sequence
  Nuclear localization signal sequence of PRPF31 protein
cggaagaagcgaggcggccgcaggtaccgcaagatgaaggag

SEQ ID NO: 17 - protein, 500 aa, Artificial Sequence
  Wild type PRPF31
  misc_feature (500)..(500): Xaa = any kind of amino acid
MSLADELLADLEEAAEEEEGGSYGEEEEEPAIEDVQEETQLDLSGDSVKTIAKLWDSKMFAEIMMKIEEYISKQAKASEVMGPVEAAPEYRVIVDANNLTVEIENELNIIHKFIRDKYSKRFPELESLVPNALDYIRTVKELGNSLDKCKNNENLQQILTNATIMVVSVTASTTQGQQLSEEELERLEEACDMALELNASKHRIYEYVESRMSFIAPNLSIIIGASTAAKIMGVAGGLTNLSKMPACNIMLLGAQRKTLSGFSSTSVLPHTGYIYHSDIVQSLPPDLRRKAARLVAAKCTLAARVDSFHESTEGKVGYELKDEIERKFDKWQEPPPVKQVKPLPAPLDGQRKKRGGRRYRKMKERLGLTEIRKQANRMSFGEIEEDAYQEDLGFSLGHLGKSGSGRVRQTQVNEATKARISKTLQRTLQKQSVVYGGKSTIRDRSSGTASSVAFTPLQGLEIVNPQAAEKKVAEANQKYFSSMAEFLKVKGEKSGLMSTX

SEQ ID NO: 18 - protein, 493 aa, Artificial Sequence
  PRPF31-sv40
  misc_feature (493)..(493): Xaa = any kind of amino acid
MSLADELLADLEEAAEEEEGGSYGEEEEEPAIEDVQEETQLDLSGDSVKTIAKLWDSKMFAEIMMKIEEYISKQAKASEVMGPVEAAPEYRVIVDANNLTVEIENELNIIHKFIRDKYSKRFPELESLVPNALDYIRTVKELGNSLDKCKNNENLQQILTNATIMVVSVTASTTQGQQLSEEELERLEEACDMALELNASKHRIYEYVESRMSFIAPNLSIIIGASTAAKIMGVAGGLTNLSKMPACNIMLLGAQRKTLSGFSSTSVLPHTGYIYHSDIVQSLPPDLRRKAARLVAAKCTLAARVDSFHESTEGKVGYELKDEIERKFDKWQEPPPVKQVKPLPAPLDGQPKKKRKVRLGLTEIRKQANRMSFGEIEEDAYQEDLGFSLGHLGKSGSGRVRQTQVNEATKARISKTLQRTLQKQSVVYGGKSTIRDRSSGTASSVAFTPLQGLEIVNPQAAEKKVAEANQKYFSSMAEFLKVKGEKSGLMSTX

SEQ ID NO: 19 - protein, 506 aa, Artificial Sequence
  PRPF31-A1
  misc_feature (506)..(506): Xaa = any kind of amino acid
MSLADELLADLEEAAEEEEGGSYGEEEEEPAIEDVQEETQLDLSGDSVKTIAKLWDSKMFAEIMMKIEEYISKQAKASEVMGPVEAAPEYRVIVDANNLTVEIENELNIIHKFIRDKYSKRFPELESLVPNALDYIRTVKELGNSLDKCKNNENLQQILTNATIMVVSVTASTTQGQQLSEEELERLEEACDMALELNASKHRIYEYVESRMSFIAPNLSIIIGASTAAKIMGVAGGLTNLSKMPACNIMLLGAQRKTLSGFSSTSVLPHTGYIYHSDIVQSLPPDLRRKAARLVAAKCTLAARVDSFHESTEGKVGYELKDEIERKFDKWQEPPPVKQVKPLPAPLDGQSSNFGPMKGGNRFFRSSGPYRLGLTEIRKQANRMSFGEIEEDAYQEDLGFSLGHLGKSGSGRVRQTQVNEATKARISKTLQRTLQKQSVVYGGKSTIRDRSSGTASSVAFTPLQGLEIVNPQAAEKKVAEANQKYFSSMAEFLKVKGEKSGLMSTX

SEQ ID NO: 20 - protein, 498 aa, Artificial Sequence
  PRPF31-TAT
  misc_feature (498)..(498): Xaa = any kind of amino acid
MSLADELLADLEEAAEEEEGGSYGEEEEEPAIEDVQEETQLDLSGDSVKTIAKLWDSKMFAEIMMKIEEYISKQAKASEVMGPVEAAPEYRVIVDANNLTVEIENELNIIHKFIRDKYSKRFPELESLVPNALDYIRTVKELGNSLDKCKNNENLQQILTNATIMVVSVTASTTQGQQLSEEELERLEEACDMALELNASKHRIYEYVESRMSFIAPNLSIIIGASTAAKIMGVAGGLTNLSKMPACNIMLLGAQRKTLSGFSSTSVLPHTGYIYHSDIVQSLPPDLRRKAARLVAAKCTLAARVDSFHESTEGKVGYELKDEIERKFDKWQEPPPVKQVKPLPAPLDGQGRKKRRQRRRAPRLGLTEIRKQANRMSFGEIEEDAYQEDLGFSLGHLGKSGSGRVRQTQVNEATKARISKTLQRTLQKQSVVYGGKSTIRDRSSGTASSVAFTPLQGLEIVNPQAAEKKVAEANQKYFSSMAEFLKVKGEKSGLMSTX

SEQ ID NO: 21 - protein, 513 aa, Artificial Sequence
  PRPF31-D
  misc_feature (513)..(513): Xaa = any kind of amino acid
MSLADELLADLEEAAEEEEGGSYGEEEEEPAIEDVQEETQLDLSGDSVKTIAKLWDSKMFAEIMMKIEEYISKQAKASEVMGPVEAAPEYRVIVDANNLTVEIENELNIIHKFIRDKYSKRFPELESLVPNALDYIRTVKELGNSLDKCKNNENLQQILTNATIMVVSVTASTTQGQQLSEEELERLEEACDMALELNASKHRIYEYVESRMSFIAPNLSIIIGASTAAKIMGVAGGLTNLSKMPACNIMLLGAQRKTLSGFSSTSVLPHTGYIYHSDIVQSLPPDLRRKAARLVAAKCTLAARVDSFHESTEGKVGYELKDEIERKFDKWQEPPPVKQVKPLPAPLDGQYGDYSNQQSGYGKVSRRGGHQNSYKPYRLGLTEIRKQANRMSFGEIEEDAYQEDLGFSLGHLGKSGSGRVRQTQVNEATKARISKTLQRTLQKQSVVYGGKSTIRDRSSGTASSVAFTPLQGLEIVNPQAAEKKVAEANQKYFSSMAEFLKVKGEKSGLMSTX

SEQ ID NO: 22 - protein, 512 aa, Artificial Sequence
  PRPF31-M
  misc_feature (512)..(512): Xaa = any kind of amino acid
MSLADELLADLEEAAEEEEGGSYGEEEEEPAIEDVQEETQLDLSGDSVKTIAKLWDSKMFAEIMMKIEEYISKQAKASEVMGPVEAAPEYRVIVDANNLTVEIENELNIIHKFIRDKYSKRFPELESLVPNALDYIRTVKELGNSLDKCKNNENLQQILTNATIMVVSVTASTTQGQQLSEEELERLEEACDMALELNASKHRIYEYVESRMSFIAPNLSIIIGASTAAKIMGVAGGLTNLSKMPACNIMLLGAQRKTLSGFSSTSVLPHTGYIYHSDIVQSLPPDLRRKAARLVAAKCTLAARVDSFHESTEGKVGYELKDEIERKFDKWQEPPPVKQVKPLPAPLDGQGEGERPAQNEKRKENIKRGGNRFEPYRLGLTEIRKQANRMSFGEIEEDAYQEDLGFSLGHLGKSGSGRVRQTQVNEATKARISKTLQRTLQKQSVVYGGKSTIRDRSSGTASSVAFTPLQGLEIVNPQAAEKKVAEANQKYFSSMAEFLKVKGEKSGLMSTX

SEQ ID NO: 23 - protein, 502 aa, Artificial Sequence
  PRPF31-NP
  misc_feature (502)..(502): Xaa = any kind of amino acid
MSLADELLADLEEAAEEEEGGSYGEEEEEPAIEDVQEETQLDLSGDSVKTIAKLWDSKMFAEIMMKIEEYISKQAKASEVMGPVEAAPEYRVIVDANNLTVEIENELNIIHKFIRDKYSKRFPELESLVPNALDYIRTVKELGNSLDKCKNNENLQQILTNATIMVVSVTASTTQGQQLSEEELERLEEACDMALELNASKHRIYEYVESRMSFIAPNLSIIIGASTAAKIMGVAGGLTNLSKMPACNIMLLGAQRKTLSGFSSTSVLPHTGYIYHSDIVQSLPPDLRRKAARLVAAKCTLAARVDSFHESTEGKVGYELKDEIERKFDKWQEPPPVKQVKPLPAPLDGQKRPAATKKAGQAKKKKRLGLTEIRKQANRMSFGEIEEDAYQEDLGFSLGHLGKSGSGRVRQTQVNEATKARISKTLQRTLQKQSVVYGGKSTIRDRSSGTASSVAFTPLQGLEIVNPQAAEKKVAEANQKYFSSMAEFLKVKGEKSGLMSTX

SEQ ID NO: 24 - protein, 505 aa, Artificial Sequence
  PRPF31-SRY
  misc_feature (505)..(505): Xaa = any kind of amino acid
MSLADELLADLEEAAEEEEGGSYGEEEEEPAIEDVQEETQLDLSGDSVKTIAKLWDSKMFAEIMMKIEEYISKQAKASEVMGPVEAAPEYRVIVDANNLTVEIENELNIIHKFIRDKYSKRFPELESLVPNALDYIRTVKELGNSLDKCKNNENLQQILTNATIMVVSVTASTTQGQQLSEEELERLEEACDMALELNASKHRIYEYVESRMSFIAPNLSIIIGASTAAKIMGVAGGLTNLSKMPACNIMLLGAQRKTLSGFSSTSVLPHTGYIYHSDIVQSLPPDLRRKAARLVAAKCTLAARVDSFHESTEGKVGYELKDEIERKFDKWQEPPPVKQVKPLPAPLDGQHREKYPNYKYRPRRKAKMLRLGLTEIRKQANRMSFGEIEEDAYQEDLGFSLGHLGKSGSGRVRQTQVNEATKARISKTLQRTLQKQSVVYGGKSTIRDRSSGTASSVAFTPLQGLEIVNPQAAEKKVAEANQKYFSSMAEFLKVKGEKSGLMSTX

SEQ ID NO: 25 - DNA, 1500 bp, Artificial Sequence
  Wild type PRPF31
atgtctctggcagatgagctcttagctgatctcgaagaggcagcagaagaggaggaaggaggaagctatggggaggaagaagaggagccagcgatcgaggatgtgcaggaggagacacagctggatctttccggggattcagtcaagaccatcgccaagctatgggatagtaagatgtttgctgagattatgatgaagattgaggagtatatcagcaagcaagccaaagcttcagaagtgatgggaccagtggaggccgcgcctgaataccgcgtcatcgtggatgccaacaacctgaccgtggagatcgaaaacgagctgaacatcatccataagttcatccgggataagtactcaaagagattccctgaactggagtccttggtccccaatgcactggattacatccgcacggtcaaggagctgggcaacagcctggacaagtgcaagaacaatgagaacctgcagcagatcctcaccaatgccaccatcatggtcgtcagcgtcaccgcctccaccacccaggggcagcagctgtcggaggaggagctggagcggctggaggaggcctgcgacatggcgctggagctgaacgcctccaagcaccgcatctacgagtatgtggagtcccggatgtccttcatcgcacccaacctgtccatcattatcggggcatccacggccgccaagatcatgggtgtggccggcggcctgaccaacctctccaagatgcccgcctgcaacatcatgctgctcggggcccagcgcaagacgctgtcgggcttctcgtctacctcagtgctgccccacaccggctacatctaccacagtgacatcgtgcagtccctgccaccggatctgcggcggaaagcggcccggctggtggccgccaagtgcacactggcagcccgtgtggacagtttccacgagagcacagaagggaaggtgggctacgaactgaaggatgagatcgagcgcaaattcgacaagtggcaggagccgccgcctgtgaagcaggtgaagccgctgcctgcgcccctggatggacagcggaagaagcgaggcggccgcaggtaccgcaagatgaaggagcggctggggctgacggagatccggaagcaggccaaccgtatgagcttcggagagatcgaggaggacgcctaccaggaggacctgggattcagcctgggccacctgggcaagtcgggcagtgggcgtgtgcggcagacacaggtaaacgaggccaccaaggccaggatctccaagacgctgcagcggaccctgcagaagcagagcgtcgtatatggcgggaagtccaccatccgcgaccgctcctcgggcacggcctccagcgtggccttcaccccactccagggcctggagattgtgaacccacaggcggcagagaagaaggtggctgaggccaaccagaagtatttctccagcatggctgagttcctcaaggtcaagggcgagaagagtggccttatgtccacctga

SEQ ID NO: 26 - DNA, 1479 bp, Artificial Sequence
  PRPF31-sv40
atgtctctggcagatgagctcttagctgatctcgaagaggcagcagaagaggaggaaggaggaagctatggggaggaagaagaggagccagcgatcgaggatgtgcaggaggagacacagctggatctttccggggattcagtcaagaccatcgccaagctatgggatagtaagatgtttgctgagattatgatgaagattgaggagtatatcagcaagcaagccaaagcttcagaagtgatgggaccagtggaggccgcgcctgaataccgcgtcatcgtggatgccaacaacctgaccgtggagatcgaaaacgagctgaacatcatccataagttcatccgggataagtactcaaagagattccctgaactggagtccttggtccccaatgcactggattacatccgcacggtcaaggagctgggcaacagcctggacaagtgcaagaacaatgagaacctgcagcagatcctcaccaatgccaccatcatggtcgtcagcgtcaccgcctccaccacccaggggcagcagctgtcggaggaggagctggagcggctggaggaggcctgcgacatggcgctggagctgaacgcctccaagcaccgcatctacgagtatgtggagtcccggatgtccttcatcgcacccaacctgtccatcattatcggggcatccacggccgccaagatcatgggtgtggccggcggcctgaccaacctctccaagatgcccgcctgcaacatcatgctgctcggggcccagcgcaagacgctgtcgggcttctcgtctacctcagtgctgccccacaccggctacatctaccacagtgacatcgtgcagtccctgccaccggatctgcggcggaaagcggcccggctggtggccgccaagtgcacactggcagcccgtgtggacagtttccacgagagcacagaagggaaggtgggctacgaactgaaggatgagatcgagcgcaaattcgacaagtggcaggagccgccgcctgtgaagcaggtgaagccgctgcctgcgcccctggatggacagcctaagaagaaaagaaaggtgcggctggggctgacggagatccggaagcaggccaaccgtatgagcttcggagagatcgaggaggacgcctaccaggaggacctgggattcagcctgggccacctgggcaagtcgggcagtgggcgtgtgcggcagacacaggtaaacgaggccaccaaggccaggatctccaagacgctgcagcggaccctgcagaagcagagcgtcgtatatggcgggaagtccaccatccgcgaccgctcctcgggcacggcctccagcgtggccttcaccccactccagggcctggagattgtgaacccacaggcggcagagaagaaggtggctgaggccaaccagaagtatttctccagcatggctgagttcctcaaggtcaagggcgagaagagtggccttatgtccacctga

SEQ ID NO: 27 - DNA, 1518 bp, Artificial Sequence
  PRPF31-A1
atgtctctggcagatgagctcttagctgatctcgaagaggcagcagaagaggaggaaggaggaagctatggggaggaagaagaggagccagcgatcgaggatgtgcaggaggagacacagctggatctttccggggattcagtcaagaccatcgccaagctatgggatagtaagatgtttgctgagattatgatgaagattgaggagtatatcagcaagcaagccaaagcttcagaagtgatgggaccagtggaggccgcgcctgaataccgcgtcatcgtggatgccaacaacctgaccgtggagatcgaaaacgagctgaacatcatccataagttcatccgggataagtactcaaagagattccctgaactggagtccttggtccccaatgcactggattacatccgcacggtcaaggagctgggcaacagcctggacaagtgcaagaacaatgagaacctgcagcagatcctcaccaatgccaccatcatggtcgtcagcgtcaccgcctccaccacccaggggcagcagctgtcggaggaggagctggagcggctggaggaggcctgcgacatggcgctggagctgaacgcctccaagcaccgcatctacgagtatgtggagtcccggatgtccttcatcgcacccaacctgtccatcattatcggggcatccacggccgccaagatcatgggtgtggccggcggcctgaccaacctctccaagatgcccgcctgcaacatcatgctgctcggggcccagcgcaagacgctgtcgggcttctcgtctacctcagtgctgccccacaccggctacatctaccacagtgacatcgtgcagtccctgccaccggatctgcggcggaaagcggcccggctggtggccgccaagtgcacactggcagcccgtgtggacagtttccacgagagcacagaagggaaggtgggctacgaactgaaggatgagatcgagcgcaaattcgacaagtggcaggagccgccgcctgtgaagcaggtgaagccgctgcctgcgcccctggatggacagtctagcaacttcggccctatgaagggcggaaaccggttctttagaagctccggcccctaccggctggggctgacggagatccggaagcaggccaaccgtatgagcttcggagagatcgaggaggacgcctaccaggaggacctgggattcagcctgggccacctgggcaagtcgggcagtgggcgtgtgcggcagacacaggtaaacgaggccaccaaggccaggatctccaagacgctgcagcggaccctgcagaagcagagcgtcgtatatggcgggaagtccaccatccgcgaccgctcctcgggcacggcctccagcgtggccttcaccccactccagggcctggagattgtgaacccacaggcggcagagaagaaggtggctgaggccaaccagaagtatttctccagcatggctgagttcctcaaggtcaagggcgagaagagtggccttatgtccacctga

SEQ ID NO: 28 - DNA, 1494 bp, Artificial Sequence
  PRPF31-TAT
atgtctctggcagatgagctcttagctgatctcgaagaggcagcagaagaggaggaaggaggaagctatggggaggaagaagaggagccagcgatcgaggatgtgcaggaggagacacagctggatctttccggggattcagtcaagaccatcgccaagctatgggatagtaagatgtttgctgagattatgatgaagattgaggagtatatcagcaagcaagccaaagcttcagaagtgatgggaccagtggaggccgcgcctgaataccgcgtcatcgtggatgccaacaacctgaccgtggagatcgaaaacgagctgaacatcatccataagttcatccgggataagtactcaaagagattccctgaactggagtccttggtccccaatgcactggattacatccgcacggtcaaggagctgggcaacagcctggacaagtgcaagaacaatgagaacctgcagcagatcctcaccaatgccaccatcatggtcgtcagcgtcaccgcctccaccacccaggggcagcagctgtcggaggaggagctggagcggctggaggaggcctgcgacatggcgctggagctgaacgcctccaagcaccgcatctacgagtatgtggagtcccggatgtccttcatcgcacccaacctgtccatcattatcggggcatccacggccgccaagatcatgggtgtggccggcggcctgaccaacctctccaagatgcccgcctgcaacatcatgctgctcggggcccagcgcaagacgctgtcgggcttctcgtctacctcagtgctgccccacaccggctacatctaccacagtgacatcgtgcagtccctgccaccggatctgcggcggaaagcggcccggctggtggccgccaagtgcacactggcagcccgtgtggacagtttccacgagagcacagaagggaaggtgggctacgaactgaaggatgagatcgagcgcaaattcgacaagtggcaggagccgccgcctgtgaagcaggtgaagccgctgcctgcgcccctggatggacagggcagaaagaagcggagacagagaagacgggcccctcggctggggctgacggagatccggaagcaggccaaccgtatgagcttcggagagatcgaggaggacgcctaccaggaggacctgggattcagcctgggccacctgggcaagtcgggcagtgggcgtgtgcggcagacacaggtaaacgaggccaccaaggccaggatctccaagacgctgcagcggaccctgcagaagcagagcgtcgtatatggcgggaagtccaccatccgcgaccgctcctcgggcacggcctccagcgtggccttcaccccactccagggcctggagattgtgaacccacaggcggcagagaagaaggtggctgaggccaaccagaagtatttctccagcatggctgagttcctcaaggtcaagggcgagaagagtggccttatgtccacctga

SEQ ID NO: 29 - DNA, 1539 bp, Artificial Sequence
  PRPF31-D
atgtctctggcagatgagctcttagctgatctcgaagaggcagcagaagaggaggaaggaggaagctatggggaggaagaagaggagccagcgatcgaggatgtgcaggaggagacacagctggatctttccggggattcagtcaagaccatcgccaagctatgggatagtaagatgtttgctgagattatgatgaagattgaggagtatatcagcaagcaagccaaagcttcagaagtgatgggaccagtggaggccgcgcctgaataccgcgtcatcgtggatgccaacaacctgaccgtggagatcgaaaacgagctgaacatcatccataagttcatccgggataagtactcaaagagattccctgaactggagtccttggtccccaatgcactggattacatccgcacggtcaaggagctgggcaacagcctggacaagtgcaagaacaatgagaacctgcagcagatcctcaccaatgccaccatcatggtcgtcagcgtcaccgcctccaccacccaggggcagcagctgtcggaggaggagctggagcggctggaggaggcctgcgacatggcgctggagctgaacgcctccaagcaccgcatctacgagtatgtggagtcccggatgtccttcatcgcacccaacctgtccatcattatcggggcatccacggccgccaagatcatgggtgtggccggcggcctgaccaacctctccaagatgcccgcctgcaacatcatgctgctcggggcccagcgcaagacgctgtcgggcttctcgtctacctcagtgctgccccacaccggctacatctaccacagtgacatcgtgcagtccctgccaccggatctgcggcggaaagcggcccggctggtggccgccaagtgcacactggcagcccgtgtggacagtttccacgagagcacagaagggaaggtgggctacgaactgaaggatgagatcgagcgcaaattcgacaagtggcaggagccgccgcctgtgaagcaggtgaagccgctgcctgcgcccctggatggacagtatggcgactacagcaaccagcagtccggctacggcaaggtgtctagacggggcggacaccagaacagctacaagccttaccggctggggctgacggagatccggaagcaggccaaccgtatgagcttcggagagatcgaggaggacgcctaccaggaggacctgggattcagcctgggccacctgggcaagtcgggcagtgggcgtgtgcggcagacacaggtaaacgaggccaccaaggccaggatctccaagacgctgcagcggaccctgcagaagcagagcgtcgtatatggcgggaagtccaccatccgcgaccgctcctcgggcacggcctccagcgtggccttcaccccactccagggcctggagattgtgaacccacaggcggcagagaagaaggtggctgaggccaaccagaagtatttctccagcatggctgagttcctcaaggtcaagggcgagaagagtggccttatgtccacctga

SEQ ID NO: 30 - DNA, 1536 bp, Artificial Sequence
  PRPF31-M
atgtctctggcagatgagctcttagctgatctcgaagaggcagcagaagaggaggaaggaggaagctatggggaggaagaagaggagccagcgatcgaggatgtgcaggaggagacacagctggatctttccggggattcagtcaagaccatcgccaagctatgggatagtaagatgtttgctgagattatgatgaagattgaggagtatatcagcaagcaagccaaagcttcagaagtgatgggaccagtggaggccgcgcctgaataccgcgtcatcgtggatgccaacaacctgaccgtggagatcgaaaacgagctgaacatcatccataagttcatccgggataagtactcaaagagattccctgaactggagtccttggtccccaatgcactggattacatccgcacggtcaaggagctgggcaacagcctggacaagtgcaagaacaatgagaacctgcagcagatcctcaccaatgccaccatcatggtcgtcagcgtcaccgcctccaccacccaggggcagcagctgtcggaggaggagctggagcggctggaggaggcctgcgacatggcgctggagctgaacgcctccaagcaccgcatctacgagtatgtggagtcccggatgtccttcatcgcacccaacctgtccatcattatcggggcatccacggccgccaagatcatgggtgtggccggcggcctgaccaacctctccaagatgcccgcctgcaacatcatgctgctcggggcccagcgcaagacgctgtcgggcttctcgtctacctcagtgctgccccacaccggctacatctaccacagtgacatcgtgcagtccctgccaccggatctgcggcggaaagcggcccggctggtggccgccaagtgcacactggcagcccgtgtggacagtttccacgagagcacagaagggaaggtgggctacgaactgaaggatgagatcgagcgcaaattcgacaagtggcaggagccgccgcctgtgaagcaggtgaagccgctgcctgcgcccctggatggacagggcgaaggcgagagacctgcccagaacgagaaaagaaaggaaaacatcaagcggggcggaaatagattcgagccctaccggctggggctgacggagatccggaagcaggccaaccgtatgagcttcggagagatcgaggaggacgcctaccaggaggacctgggattcagcctgggccacctgggcaagtcgggcagtgggcgtgtgcggcagacacaggtaaacgaggccaccaaggccaggatctccaagacgctgcagcggaccctgcagaagcagagcgtcgtatatggcgggaagtccaccatccgcgaccgctcctcgggcacggcctccagcgtggccttcaccccactccagggcctggagattgtgaacccacaggcggcagagaagaaggtggctgaggccaaccagaagtatttctccagcatggctgagttcctcaaggtcaagggcgagaagagtggccttatgtccacctga

SEQ ID NO: 31 - DNA, 1506 bp, Artificial Sequence
  PRPF31-NP
atgtctctggcagatgagctcttagctgatctcgaagaggcagcagaagaggaggaaggaggaagctatggggaggaagaagaggagccagcgatcgaggatgtgcaggaggagacacagctggatctttccggggattcagtcaagaccatcgccaagctatgggatagtaagatgtttgctgagattatgatgaagattgaggagtatatcagcaagcaagccaaagcttcagaagtgatgggaccagtggaggccgcgcctgaataccgcgtcatcgtggatgccaacaacctgaccgtggagatcgaaaacgagctgaacatcatccataagttcatccgggataagtactcaaagagattccctgaactggagtccttggtccccaatgcactggattacatccgcacggtcaaggagctgggcaacagcctggacaagtgcaagaacaatgagaacctgcagcagatcctcaccaatgccaccatcatggtcgtcagcgtcaccgcctccaccacccaggggcagcagctgtcggaggaggagctggagcggctggaggaggcctgcgacatggcgctggagctgaacgcctccaagcaccgcatctacgagtatgtggagtcccggatgtccttcatcgcacccaacctgtccatcattatcggggcatccacggccgccaagatcatgggtgtggccggcggcctgaccaacctctccaagatgcccgcctgcaacatcatgctgctcggggcccagcgcaagacgctgtcgggcttctcgtctacctcagtgctgccccacaccggctacatctaccacagtgacatcgtgcagtccctgccaccggatctgcggcggaaagcggcccggctggtggccgccaagtgcacactggcagcccgtgtggacagtttccacgagagcacagaagggaaggtgggctacgaactgaaggatgagatcgagcgcaaattcgacaagtggcaggagccgccgcctgtgaagcaggtgaagccgctgcctgcgcccctggatggacagaaaagacctgctgccaccaagaaggccggccaggccaagaagaaaaagcggctggggctgacggagatccggaagcaggccaaccgtatgagcttcggagagatcgaggaggacgcctaccaggaggacctgggattcagcctgggccacctgggcaagtcgggcagtgggcgtgtgcggcagacacaggtaaacgaggccaccaaggccaggatctccaagacgctgcagcggaccctgcagaagcagagcgtcgtatatggcgggaagtccaccatccgcgaccgctcctcgggcacggcctccagcgtggccttcaccccactccagggcctggagattgtgaacccacaggcggcagagaagaaggtggctgaggccaaccagaagtatttctccagcatggctgagttcctcaaggtcaagggcgagaagagtggccttatgtccacctga

SEQ ID NO: 32 - DNA, 1515 bp, Artificial Sequence
  PRPF31-SRY
atgtctctggcagatgagctcttagctgatctcgaagaggcagcagaagaggaggaaggaggaagctatggggaggaagaagaggagccagcgatcgaggatgtgcaggaggagacacagctggatctttccggggattcagtcaagaccatcgccaagctatgggatagtaagatgtttgctgagattatgatgaagattgaggagtatatcagcaagcaagccaaagcttcagaagtgatgggaccagtggaggccgcgcctgaataccgcgtcatcgtggatgccaacaacctgaccgtggagatcgaaaacgagctgaacatcatccataagttcatccgggataagtactcaaagagattccctgaactggagtccttggtccccaatgcactggattacatccgcacggtcaaggagctgggcaacagcctggacaagtgcaagaacaatgagaacctgcagcagatcctcaccaatgccaccatcatggtcgtcagcgtcaccgcctccaccacccaggggcagcagctgtcggaggaggagctggagcggctggaggaggcctgcgacatggcgctggagctgaacgcctccaagcaccgcatctacgagtatgtggagtcccggatgtccttcatcgcacccaacctgtccatcattatcggggcatccacggccgccaagatcatgggtgtggccggcggcctgaccaacctctccaagatgcccgcctgcaacatcatgctgctcggggcccagcgcaagacgctgtcgggcttctcgtctacctcagtgctgccccacaccggctacatctaccacagtgacatcgtgcagtccctgccaccggatctgcggcggaaagcggcccggctggtggccgccaagtgcacactggcagcccgtgtggacagtttccacgagagcacagaagggaaggtgggctacgaactgaaggatgagatcgagcgcaaattcgacaagtggcaggagccgccgcctgtgaagcaggtgaagccgctgcctgcgcccctggatggacagcacagagagaaataccccaactacaagtaccggcctagaagaaaggccaagatgctgcggctggggctgacggagatccggaagcaggccaaccgtatgagcttcggagagatcgaggaggacgcctaccaggaggacctgggattcagcctgggccacctgggcaagtcgggcagtgggcgtgtgcggcagacacaggtaaacgaggccaccaaggccaggatctccaagacgctgcagcggaccctgcagaagcagagcgtcgtatatggcgggaagtccaccatccgcgaccgctcctcgggcacggcctccagcgtggccttcaccccactccagggcctggagattgtgaacccacaggcggcagagaagaaggtggctgaggccaaccagaagtatttctccagcatggctgagttcctcaaggtcaagggcgagaagagtggccttatgtccacctga

SEQ ID NO: 33 - DNA, 653 bp, Artificial Sequence
  RHO minigene reporter gene
gctgttcccaagtccctcacaggcagggtctccctacctgcctgtcctcaggtacatccccgagggcctgcagtgctcgtgtggaatcgactactacacgctcaagccggaggtcaacaacgagtcttttgtcatctacatgttcgtggtccacttcaccatccccatgattatcatctttttctgctatgggcagctcgtcttcaccgtcaaggaggtacgggccggggggtgggcggcctcacggctctgagggtccagcccccagcatgcatctgcggctcctgctccctggaggagccatggtctggacccgggtcccgtgtcctgcaggccgctgcccagcagcaggagtcagccaccacacagaaggcagagaaggaggtcacccgcatggtcatcatcatggtcatcgctttcctgatctgctgggtgccctacgccagcgtggcattctacatcttcacccaccagggctccaacttcggtcccatcttcatgaccatcccagcgttctttgccaagagcgccgccatctacaaccctgtcatctatatcatgatgaacaagcaggtgcctactgcgggtgggagggccccagtgccccaggccacaggcgctgcctgccaaggacaagctacttcccagggcag

SEQ ID NO: 34 - DNA, 711 bp, Artificial Sequence
  Nucleic acid molecule encoding Mcherry
atggtgagcaagggcgaggaggataacatggccatcatcaaggagttcatgcgcttcaaggtgcacatggagggctccgtgaacggccacgagttcgagatcgagggcgagggcgagggccgcccctacgagggcacccagaccgccaagctgaaggtgaccaagggtggccccctgcccttcgcctgggacatcctgtcccctcagttcatgtacggctccaaggcctacgtgaagcaccccgccgacatccccgactacttgaagctgtccttccccgagggcttcaagtgggagcgcgtgatgaacttcgaggacggcggcgtggtgaccgtgacccaggactcctccctgcaggacggcgagttcatctacaaggtgaagctgcgcggcaccaacttcccctccgacggccccgtaatgcagaagaagaccatgggctgggaggcctcctccgagcggatgtaccccgaggacggcgccctgaagggcgagatcaagcagaggctgaagctgaaggacggcggccactacgacgctgaggtcaagaccacctacaaggccaagaagcccgtgcagctgcccggcgcctacaacgtcaacatcaagttggacatcacctcccacaacgaggactacaccatcgtggaacagtacgaacgcgccgagggccgccactccaccggcggcatggacgagctgtacaagtag

SEQ ID NO: 35 - protein, 52 aa, Artificial Sequence
  NOSIC domain of PRPF31
IVDANNLTVEIENELNIIHKFIRDKYSKRFPELESLVPNALDYIRTVKELGN

SEQ ID NO: 36 - protein, 145 aa, Artificial Sequence
  NOP domain of PRPF31
ACDMALELNASKHRIYEYVESRMSFIAPNLSIIIGASTAAKIMGVAGGLTNLSKMPACNIMLLGAQRKTLSGFSSTSVLPHTGYIYHSDIVQSLPPDLRRKAARLVAAKCTLAARVDSFHESTEGKVGYELKDEIERKFDKWQEP